European Patent Application EP 4 722 361 A1, published April 8, 2026. Title: 用于制备环状RNA的载体和方法. Applicant: 南京金斯瑞生物科技有限公司. Application CN. The sequence listing filed with the application follows.

SEQUENCE LISTING (96 sequences)

SEQ ID NO: 1 - DNA, 19 bp, synthetic construct
  source 1..19: mol_type = other DNA
taatacgactcactatagg

SEQ ID NO: 2 - DNA, 20 bp, synthetic construct
  source 1..20: mol_type = other DNA
ccgtcgattgtccactggtc

SEQ ID NO: 3 - DNA, 183 bp, synthetic construct
  source 1..183: mol_type = other DNA
aacaatagatgacttacaactaatcggaaggtgcagagactcgacgggagctaccctaacgtcaagacgagggtaaagagagagtccaattctcaaagccaataggcagtagcgaaagctgcaagagaatgaaaatccgttgaccttaaacggtcgtgtgggttcaagtccctccacccccac

SEQ ID NO: 4 - DNA, 69 bp, synthetic construct
  source 1..69: mol_type = other DNA
gccggaaacgcaatagccgaaaaacaaaaaacaaaaaaaaaaaaaaaaaaaaaaaaaaaaaaaaaaaaa

SEQ ID NO: 5 - DNA, 741 bp, synthetic construct
  source 1..741: mol_type = other DNA
ttaaaacagcctgtgggttgatcccacccacaggcccattgggcgctagcactctggtatcacggtacctttgtgcgcctgttttataccccctcccccaactgtaacttagaagtaacacacaccgatcaacagtcagcgtggcacaccagccacgttttgatcaagcacttctgttaccccggactgagtatcaatagactgctcacgcggttgaaggagaaagcgttcgttatccggccaactacttcgaaaaacctagtaacaccgtggaagttgcagagtgtttcgctcagcactaccccagtgtagatcaggtcgatgagtcaccgcattccccacgggcgaccgtggcggtggctgcgttggcggcctgcccatggggaaacccatgggacgctctaatacagacatggtgcgaagagtctattgagctagttggtagtcctccggcccctgaatgcggctaatcctaactgcggagcacacaccctcaagccagagggcagtgtgtcgtaacgggcaactctgcagcggaaccgactactttgggtgtccgtgtttcattttattcctatactggctgcttatggtgacaattgagagatcgttaccatatagctattggattggccatccggtgactaatagagctattatatatccctttgttgggtttataccacttagcttgaaagaggttaaaacattacaattcattgttaagttgaatacagcaaa

SEQ ID NO: 6 - DNA, 1653 bp, synthetic construct
  source 1..1653: mol_type = other DNA
atggaagacgccaaaaacataaagaaaggcccggcgccattctatccgctggaagatggaaccgctggagagcaactgcataaggctatgaagagatacgccctggttcctggaacaattgcttttacagatgcacatatcgaggtggacatcacttacgctgagtacttcgaaatgtccgttcggttggcagaagctatgaaacgatatgggctgaatacaaatcacagaatcgtcgtatgcagtgaaaactctcttcaattctttatgccggtgttgggcgcgttatttatcggagttgcagttgcgcccgcgaacgacatttataatgaacgtgaattgctcaacagtatgggcatttcgcagcctaccgtggtgttcgtttccaaaaaggggttgcaaaaaattttgaacgtgcaaaaaaagctcccaatcatccaaaaaattattatcatggattctaaaacggattaccagggatttcagtcgatgtacacgttcgtcacatctcatctacctcccggttttaatgaatacgattttgtgccagagtccttcgatagggacaagacaattgcactgatcatgaactcctctggatctactggtctgcctaaaggtgtcgctctgcctcatagaactgcctgcgtgagattctcgcatgccagagatcctatttttggcaatcaaatcattccggatactgcgattttaagtgttgttccattccatcacggttttggaatgtttactacactcggatatttgatatgtggatttcgagtcgtcttaatgtatagatttgaagaagagctgtttctgaggagccttcaggattacaagattcaaagtgcgctgctggtgccaaccctattctccttcttcgccaaaagcactctgattgacaaatacgatttatctaatttacacgaaattgcttctggtggcgctcccctctctaaggaagtcggggaagcggttgccaagaggttccatctgccaggtatcaggcaaggatatgggctcactgagactacatcagctattctgattacacccgagggggatgataaaccgggcgcggtcggtaaagttgttccattttttgaagcgaaggttgtggatctggataccgggaaaacgctgggcgttaatcaaagaggcgaactgtgtgtgagaggtcctatgattatgtccggttatgtaaacaatccggaagcgaccaacgccttgattgacaaggatggatggctacattctggagacatagcttactgggacgaagacgaacacttcttcatcgttgaccgcctgaagtctctgattaagtacaaaggctatcaggtggctcccgctgaattggaatccatcttgctccaacaccccaacatcttcgacgcaggtgtcgcaggtcttcccgacgatgacgccggtgaacttcccgccgccgttgttgttttggagcacggaaagacgatgacggaaaaagagatcgtggattacgtcgccagtcaagtaacaaccgcgaaaaagttgcgcggaggagttgtgtttgtggacgaagtaccgaaaggtcttaccggaaaactcgacgcaagaaaaatcagagagatcctcataaaggccaagaagggcggaaagatcgccgtgtaa

SEQ ID NO: 7 - DNA, 558 bp, synthetic construct
  source 1..558: mol_type = other DNA
atgggagtcaaagttctgtttgccctgatctgcatcgctgtggccgaggccaagcccaccgagaacaacgaagacttcaacatcgtggccgtggccagcaacttcgcgaccacggatctcgatgctgaccgcgggaagttgcccggcaagaagctgccgctggaggtgctcaaagagatggaagccaatgcccggaaagctggctgcaccaggggctgtctgatctgcctgtcccacatcaagtgcacgcccaagatgaagaagttcatcccaggacgctgccacacctacgaaggcgacaaagagtccgcacagggcggcataggcgaggcgatcgtcgacattcctgagattcctgggttcaaggacttggagcccatggagcagttcatcgcacaggtcgatctgtgtgtggactgcacaactggctgcctcaaagggcttgccaacgtgcagtgttctgacctgctcaagaagtggctgccgcaacgctgtgcgacctttgccagcaagatccagggccaggtggacaagatcaagggggccggtggtgactaa

SEQ ID NO: 8 - DNA, 720 bp, synthetic construct
  source 1..720: mol_type = other DNA
atggtgagcaagggcgaggagctgttcaccggggtggtgcccatcctggtcgagctggacggcgacgtaaacggccacaagttcagcgtgtccggcgagggcgagggcgatgccacctacggcaagctgaccctgaagttcatctgcaccaccggcaagctgcccgtgccctggcccaccctcgtgaccaccctgacctacggcgtgcagtgcttcagccgctaccccgaccacatgaagcagcacgacttcttcaagtccgccatgcccgaaggctacgtccaggagcgcaccatcttcttcaaggacgacggcaactacaagacccgcgccgaggtgaagttcgagggcgacaccctggtgaaccgcatcgagctgaagggcatcgacttcaaggaggacggcaacatcctggggcacaagctggagtacaactacaacagccacaacgtctatatcatggccgacaagcagaagaacggcatcaaggtgaacttcaagatccgccacaacatcgaggacggcagcgtgcagctcgccgaccactaccagcagaacacccccatcggcgacggccccgtgctgctgcccgacaaccactacctgagcacccagtccgccctgagcaaagaccccaacgagaagcgcgatcacatggtcctgctggagttcgtgaccgccgccgggatcactctcggcatggacgagctgtacaagtaa

SEQ ID NO: 9 - DNA, 39 bp, synthetic construct
  source 1..39: mol_type = other DNA
aaaaaacaaaaaacaaaacggctattatgcgttaccggc

SEQ ID NO: 10 - DNA, 132 bp, synthetic construct
  source 1..132: mol_type = other DNA
gagacgctacggacttaaataattgagccttaaagaagaaattctttaagtggatgctctcaaactcagggaaacctaaatctagttatagacaaggcaatcctgagccaagccgaagtagtaattagtaag

SEQ ID NO: 11 - DNA, 19 bp, synthetic construct
  source 1..19: mol_type = other DNA
accagtggacaatcgacgg

SEQ ID NO: 12 - DNA, 2317 bp, synthetic construct
  source 1..2317: mol_type = other DNA
tcgcgcgtttcggtgatgacggtgaaaacctctgacacatgcagctcccggacgtcattgtcgatctccccatgcgagagtagggaactgccaggcatcaaataaaacgaaaggctcagtcgaaagactgggcctttcgttttatctgttgtttgtcggtgaacgctctcctgagtaggacaaatccgccgggagcggatttgaacgttgcgaagcaacggcccggagggtggcgggcaggacgcccgccataaactgccaggcatcaaattaagcagaaggccatcctgacggatggcctttttgcgtttctacaaactctctctggctaactagagaacccactgcttactggcttatcgaaatgctagcgtttaaacttaagcttggtaccgagctcggatcctctagagggcccgtttaaacccgctgatcagcctcgactctagcttggattctcaccaataaaaaacgcccggcggcaaccgagcgttctgaacaaatccagatggagttctgaggtcattactggatctatcaacaggagtccaagctcagatcattgtcacatgtgagcaaaaggccagcaaaaggccaggaaccgtaaaaaggccgcgttgctggcgtttttccataggctccgcccccctgacgagcatcacaaaaatcgacgctcaagtcagaggtggcgaaacccgacaggactataaagataccaggcgtttccccctggaagctccctcgtgcgctctcctgttccgaccctgccgcttaccggatacctgtccgcctttctcccttcgggaagcgtggcgctttctcatagctcacgctgtaggtatctcagttcggtgtaggtcgttcgctccaagctgggctgtgtgcacgaaccccccgttcagcccgaccgctgcgccttatccggtaactatcgtcttgagtccaacccggtaagacacgacttatcgccactggcagcagccactggtaacaggattagcagagcgaggtatgtaggcggtgctacagagttcttgaagtggtggcctaactacggctacactagaagaacagtatttggtatctgcgctctgctgaagccagttaccttcggaaaaagagttggtagctcttgatccggcaaacaaaccaccgctggtagcggtggtttttttgtttgcaagcagcagattacgcgcagaaaaaaaggatctcaagaagatcctttgatcttttctacggggtctgacgctcagtggaacgaaaactcacgttaagggattttggtcatgagattatcaaaaaggatcttcacctagatccttttaaattaaaaatgaagttttaaatcaagcccaatctgaataatgttacaaccaattaaccaattctgattagaaaaactcatcgagcatcaaatgaaactgcaatttattcatatcaggattatcaataccatatttttgaaaaagccgtttctgtaatgaaggagaaaactcaccgaggcagttccataggatggcaagatcctggtatcggtctgcgattccgactcgtccaacatcaatacaacctattaatttcccctcgtcaaaaataaggttatcaagtgagaaatcaccatgagtgacgactgaatccggtgagaatggcaaaagtttatgcatttctttccagacttgttcaacaggccagccattacgctcgtcatcaaaatcactcgcatcaaccaaaccgttattcattcgtgattgcgcctgagcgaggcgaaatacgcgatcgctgttaaaaggacaattacaaacaggaatcgaatgcaaccggcgcaggaacactgccagcgcatcaacaatattttcacctgaatcaggatattcttctaatacctggaatgctgtttttccggggatcgcagtggtgagtaaccatgcatcatcaggagtacggataaaatgcttgatggtcggaagaggcataaattccgtcagccagtttagtctgaccatctcatctgtaacatcattggcaacgctacctttgccatgtttcagaaacaactctggcgcatcgggcttcccatacaagcgatagattgtcgcacctgattgcccgacattatcgcgagcccatttatacccatataaatcagcatccatgttggaatttaatcgcggcctcgacgtttcccgttgaatatggctcataacaccccttgtattactgtttatgtaagcagacagttttattgttcatgatgatatatttttatcttgtgcaatgtaacatcagagattttgagacacgggccagagctgca

SEQ ID NO: 13 - DNA, 51 bp, synthetic construct
  source 1..51: mol_type = other DNA
gcccgggcggcctcagtgagcgagcgagcgcgcagagagggagtggccaac

SEQ ID NO: 14 - DNA, 73 bp, synthetic construct
  source 1..73: mol_type = other DNA
gttggccactccctctctgcgcgctcgctcgctcactgaggccgggcgaccaaaggtcgcccgacgcccgggc

SEQ ID NO: 15 - DNA, 33 bp, synthetic construct
  source 1..33: mol_type = other DNA
ggtccccaggcctcagtgagtgagtgagtgagc

SEQ ID NO: 16 - DNA, 55 bp, synthetic construct
  source 1..55: mol_type = other DNA
gctcactcactcactcactgaggcctgcagagcaaagctctgcagtctggggacc

SEQ ID NO: 17 - DNA, 100 bp, synthetic construct
  source 1..100: mol_type = other DNA
atggtgagcaagggcgaggagctgttcaccggggtggtgcccatcctggtcgagctggacggcgacgtaaacggccacaagttcagcgtgtctggcgagg

SEQ ID NO: 18 - DNA, 367 bp, Bacillus anthracis
  source 1..367: mol_type = genomic DNA
ttggggttatgttcggaaatcaactacaagttgcttaatcgtaaagattaaggagtttaccatgggtttcccttgctagtgatagcatgttaaaaaaccttgtgaaccttattgcctaagggtgtaactattcatatagttgctaacggtgaagcccaccattattcagggtaataccgtgccaagctccatagtgatatggggaaggtgtagagactaccgaaaaggacttttagttaactgagtagggtacggcagatgataggctactgctggaagtgcaaggctctctgtaaagagatgaagagatagtccggactatagagatggaaaatctatagatagtgccagaaacaactccaggtgg

SEQ ID NO: 19 - DNA, 328 bp, Coxiella burnetii
  source 1..328: mol_type = genomic DNA
taaacggcggccgtaactataaattaaccgttgtagttacgtaaataaacttggctatatgctggaaactccgagtatcctccagtactcatctcaactaaaattgaggtagtaaaaatctgcgaggtgcggacaatcagcaggaaagactaatctttttgattagaatcctcagagactaatacgccgagcgtacttagaaaaaatccattctaagtgtgatgatagagtccgatctctatagcgatatagagggttttcaaaagaaacctgttaatcattatcccatgattaacataacgtcaataaacggtcctaaggtagcgaa

SEQ ID NO: 20 - DNA, 735 bp, Synechocystis sp.
  source 1..735: mol_type = genomic DNA
aagcgacgcgggatagagcagtctggtagctcgtcgggctcaggtcgcaagatgtaaaccatgagcactaagcttaagggtgacattgcagagcaagccgccattcttcgtgcattgaagcttggttggggggttctgaagccattgggagaccgtctttcttacgatttggtctttgatgtcgaagggatccttctgaaggtgcaggttaaaagctcctggttcagcgaaaagactggcaactatgttgttgacaatcgcagaacaaggacaaacagaagaaacattgttagatctccttatcgtgggaatgactttgattttgctgttgcctacgtcgaagaacttgagctgttttacgtcttcccggttgatgtctttatcagttacggcagtgaaattcacctggtcgaaactgataagcgtcagagaaaaccaaggtcattcggttaccgagaggcttggcatctcatcttgcaaaaaggggctgcgcaaaaggaaacttctgcgtgattatctctcaaattcggggaagcctttcaaatggtaatcccgagccaaacctaggaatgcttggtgtttctgggaaggtgtagagacttaatgggagacaccctaacagaaaagctgagggtgaagagaaagtccagaccacaaactgacagagtcaggcagtgaaaactgtagttggtaagcataacccgaaggtcggtggttcaaatccgcctcccgcca

SEQ ID NO: 21 - DNA, 779 bp, Thermotoga naphthophila
  source 1..779: mol_type = genomic DNA
ccccggtaaacggcggccgtaactataacggtcctaaggtagcattcgctgcctgcccacagggaaacctgtggggcaatacccggctgtatgcgggaaagcccttagagcccttcctacctgggggctgcggccagcccaggtaaaaatggaagggattgggtaatccgcaggaaaccccgatgagggggatcctcagagactgtacgccgggcatccagtccccgtgagaaggggtggaaatcttggatctcaagcctgattgggttgttggattcgtcgatggtgaaggttgtttctacgtgggtgttaatagaaatcgcaccatgaagacaggttaccaagttctccctgaattcaggattgttcagcatgaaagggatatacagattctgtacgcattgaagaagttctttgggtgcggtgttgtacgaaaaaaccacgatgatcgatatgaacttcggatccggaagaagtcttgcttgaagaaagtagtggaattcttcgaaaagcaccctctgaaaacgaagaagaacgttgacttcaagaagttcagaagaataatcctgatgatggaacggggagaacacctgacgaaagaaggtctaatcaagatcttagaaatcgccatggaaatgaacacaggtaaccacgagagactgcgacgagtccttgaagagatccggggactggatgaagatacagtccacccccattccgaaaggatgggataagggtgagcgaaattccttgtcgggtaagttccgacctgcatgaat

SEQ ID NO: 22 - DNA, 215 bp, Phormidium sp.
  source 1..215: mol_type = genomic DNA
agaaastgcgccttactggagaaatcctttaagtgacckctctcaaattcagggaaacctaactctggcaacagacaaggcaatcctgagccaagccgaaatttcggaaggtgcagagactcgacgggagctaccctaacgtaaagccgagggtaaagggagagtccaattctcaaagcctaattatagggcagcagcgaaagttgcggagaatg

SEQ ID NO: 23 - DNA, 100 bp, synthetic construct
  source 1..100: mol_type = other DNA
cctacggcaagctgaccctgaagttcatctgcaccaccggcaagctgcccgtgccctggcccaccctcgtgaccaccctgacctacggcgtgcagtgctt

SEQ ID NO: 24 - DNA, 19 bp, synthetic construct
  source 1..19: mol_type = other DNA
gatggtgagcaagggcgag

SEQ ID NO: 25 - DNA, 19 bp, synthetic construct
  source 1..19: mol_type = other DNA
caagcactgcacgccgtag

SEQ ID NO: 26 - DNA, 20 bp, synthetic construct
  source 1..20: mol_type = other DNA
aatccggaagcgaccaacgc

SEQ ID NO: 27 - DNA, 20 bp, synthetic construct
  source 1..20: mol_type = other DNA
ggggccggaggactaccaac

SEQ ID NO: 28 - DNA, 20 bp, synthetic construct
  source 1..20: mol_type = other DNA
gttgcccggcaagaagctgc

SEQ ID NO: 29 - DNA, 118 bp, synthetic construct
  source 1..118: mol_type = other DNA
aacggctattatgcgttaccggcgagacgctacggacttaaaatccgttgaccttaaacggtcgtgtgggttcaagtccctccacccccacgccggaaacgcaatagccgaaaaacaa

SEQ ID NO: 30 - DNA, 101 bp, synthetic construct
  source 1..101: mol_type = other DNA
gcgacgtaaacggccacaagttcagcgtgtctggcgaggagaaaactgagccttagtggagaaatccgctaagtggaagctctcaaactcagggaaaccta

SEQ ID NO: 31 - DNA, 93 bp, synthetic construct
  source 1..93: mol_type = other DNA
acaagttcagcgtgtctggcgaggtaaacggcggccgtaactataacggtcctaaggtagcgaacctacggcaagctgaccctgaagttcatc

SEQ ID NO: 32 - DNA, 99 bp, synthetic construct
  source 1..99: mol_type = other DNA
acggccacaagttcagcgtgtctggcgaggttggggttatgttcggaaatccagaaacaactccaggtggcctacggcaagctgaccctgaagttcatc

SEQ ID NO: 33 - DNA, 126 bp, synthetic construct
  source 1..126: mol_type = other DNA
tcagcgtgtctggcgaggaagcgacgcgggatagagcagtctggtagctcgtcgggctcataacccgaaggtcggtggttcaaatccgcctcccgccacctacggcaagctgaccctgaagttcat

SEQ ID NO: 34 - DNA, 122 bp, synthetic construct
  source 1..122: mol_type = other DNA
agttcagcgtgtctggcgaggccccggtaaacggcggccgtaactataacggtcctaaggtagcgaaattccttgtcgggtaagttccgacctgcatgaatcctacggcaagctgaccctga

SEQ ID NO: 35 - DNA, 117 bp, synthetic construct
  source 1..117: mol_type = other DNA
aaaaaacaaaaaacaaaacggctattatgcgttaccggctaaacggcggccgtaactataacggtcctaaggtagcgaagccggaaacgcaatagccgaaaaacaaaaaacaaaaaa

SEQ ID NO: 36 - DNA, 117 bp, synthetic construct
  source 1..117: mol_type = other DNA
aaaaaacaaaaaacaaaacggctattatgcgttaccggcttggggttatgttcggaaatccagaaacaactccaggtgggccggaaacgcaatagccgaaaaacaaaaaacaaaaaa

SEQ ID NO: 37 - DNA, 123 bp, synthetic construct
  source 1..123: mol_type = other DNA
aaacggctattatgcgttaccggcaagcgacgcgggatagagcagtctggtagctcgtcgggctcataacccgaaggtcggtggttcaaatccgcctcccgccagccggaaacgcaatagccg

SEQ ID NO: 38 - DNA, 135 bp, synthetic construct
  source 1..135: mol_type = other DNA
aaaacggctattatgcgttaccggcccccggtaaacggcggccgtaactataacggtcctaaggtagcgaaattccttgtcgggtaagttccgacctgcatgaatgccggaaacgcaatagccgaaaaacaaaaa

SEQ ID NO: 39 - DNA, 234 bp, synthetic construct
  source 1..234: mol_type = other DNA
atatagttgctaacggtgaagcccaccattattcagggtaataccgtgccaagctccatagtgatatggggaaggtgtagagactaccgaaaaggacttttagttaactgagtagggtacggcagatgataggctactgctggaagtgcaaggctctctgtaaagagatgaagagatagtccggactatagagatggaaaatctatagatagtgccagaaacaactccaggtgg

SEQ ID NO: 40 - DNA, 133 bp, synthetic construct
  source 1..133: mol_type = other DNA
ttggggttatgttcggaaatcaactacaagttgcttaatcgtaaagattaaggagtttaccatgggtttcccttgctagtgatagcatgttaaaaaaccttgtgaaccttattgcctaagggtgtaactattc

SEQ ID NO: 41 - DNA, 172 bp, synthetic construct
  source 1..172: mol_type = other DNA
gatatggggaaggtgtagagactaccgaaaaggacttttagttaactgagtagggtacggcagatgataggctactgctggaagtgcaaggctctctgtaaagagatgaagagatagtccggactatagagatggaaaatctatagatagtgccagaaacaactccaggtgg

SEQ ID NO: 42 - DNA, 195 bp, synthetic construct
  source 1..195: mol_type = other DNA
ttggggttatgttcggaaatcaactacaagttgcttaatcgtaaagattaaggagtttaccatgggtttcccttgctagtgatagcatgttaaaaaaccttgtgaaccttattgcctaagggtgtaactattcatatagttgctaacggtgaagcccaccattattcagggtaataccgtgccaagctccatagt

SEQ ID NO: 43 - DNA, 73 bp, synthetic construct
  source 1..73: mol_type = other DNA
aaagagatgaagagatagtccggactatagagatggaaaatctatagatagtgccagaaacaactccaggtgg

SEQ ID NO: 44 - DNA, 294 bp, synthetic construct
  source 1..294: mol_type = other DNA
ttggggttatgttcggaaatcaactacaagttgcttaatcgtaaagattaaggagtttaccatgggtttcccttgctagtgatagcatgttaaaaaaccttgtgaaccttattgcctaagggtgtaactattcatatagttgctaacggtgaagcccaccattattcagggtaataccgtgccaagctccatagtgatatggggaaggtgtagagactaccgaaaaggacttttagttaactgagtagggtacggcagatgataggctactgctggaagtgcaaggctctctgt

SEQ ID NO: 45 - DNA, 171 bp, synthetic construct
  source 1..171: mol_type = other DNA
tttgattagaatcctcagagactaatacgccgagcgtacttagaaaaaatccattctaagtgtgatgatagagtccgatctctatagcgatatagagggttttcaaaagaaacctgttaatcattatcccatgattaacataacgtcaataaacggtcctaaggtagcgaa

SEQ ID NO: 46 - DNA, 157 bp, synthetic construct
  source 1..157: mol_type = other DNA
taaacggcggccgtaactataaattaaccgttgtagttacgtaaataaacttggctatatgctggaaactccgagtatcctccagtactcatctcaactaaaattgaggtagtaaaaatctgcgaggtgcggacaatcagcaggaaagactaatctt

SEQ ID NO: 47 - DNA, 228 bp, synthetic construct
  source 1..228: mol_type = other DNA
aaattgaggtagtaaaaatctgcgaggtgcggacaatcagcaggaaagactaatctttttgattagaatcctcagagactaatacgccgagcgtacttagaaaaaatccattctaagtgtgatgatagagtccgatctctatagcgatatagagggttttcaaaagaaacctgttaatcattatcccatgattaacataacgtcaataaacggtcctaaggtagcgaa

SEQ ID NO: 48 - DNA, 100 bp, synthetic construct
  source 1..100: mol_type = other DNA
taaacggcggccgtaactataaattaaccgttgtagttacgtaaataaacttggctatatgctggaaactccgagtatcctccagtactcatctcaacta

SEQ ID NO: 49 - DNA, 623 bp, synthetic construct
  source 1..623: mol_type = other DNA
cattgaagcttggttggggggttctgaagccattgggagaccgtctttcttacgatttggtctttgatgtcgaagggatccttctgaaggtgcaggttaaaagctcctggttcagcgaaaagactggcaactatgttgttgacaatcgcagaacaaggacaaacagaagaaacattgttagatctccttatcgtgggaatgactttgattttgctgttgcctacgtcgaagaacttgagctgttttacgtcttcccggttgatgtctttatcagttacggcagtgaaattcacctggtcgaaactgataagcgtcagagaaaaccaaggtcattcggttaccgagaggcttggcatctcatcttgcaaaaaggggctgcgcaaaaggaaacttctgcgtgattatctctcaaattcggggaagcctttcaaatggtaatcccgagccaaacctaggaatgcttggtgtttctgggaaggtgtagagacttaatgggagacaccctaacagaaaagctgagggtgaagagaaagtccagaccacaaactgacagagtcaggcagtgaaaactgtagttggtaagcataacccgaaggtcggtggttcaaatccgcctcccgcca

SEQ ID NO: 50 - DNA, 112 bp, synthetic construct
  source 1..112: mol_type = other DNA
aagcgacgcgggatagagcagtctggtagctcgtcgggctcaggtcgcaagatgtaaaccatgagcactaagcttaagggtgacattgcagagcaagccgccattcttcgtg

SEQ ID NO: 51 - DNA, 437 bp, synthetic construct
  source 1..437: mol_type = other DNA
cttatcgtgggaatgactttgattttgctgttgcctacgtcgaagaacttgagctgttttacgtcttcccggttgatgtctttatcagttacggcagtgaaattcacctggtcgaaactgataagcgtcagagaaaaccaaggtcattcggttaccgagaggcttggcatctcatcttgcaaaaaggggctgcgcaaaaggaaacttctgcgtgattatctctcaaattcggggaagcctttcaaatggtaatcccgagccaaacctaggaatgcttggtgtttctgggaaggtgtagagacttaatgggagacaccctaacagaaaagctgagggtgaagagaaagtccagaccacaaactgacagagtcaggcagtgaaaactgtagttggtaagcataacccgaaggtcggtggttcaaatccgcctcccgcca

SEQ ID NO: 52 - DNA, 298 bp, synthetic construct
  source 1..298: mol_type = other DNA
aagcgacgcgggatagagcagtctggtagctcgtcgggctcaggtcgcaagatgtaaaccatgagcactaagcttaagggtgacattgcagagcaagccgccattcttcgtgcattgaagcttggttggggggttctgaagccattgggagaccgtctttcttacgatttggtctttgatgtcgaagggatccttctgaaggtgcaggttaaaagctcctggttcagcgaaaagactggcaactatgttgttgacaatcgcagaacaaggacaaacagaagaaacattgttagatctc

SEQ ID NO: 53 - DNA, 410 bp, synthetic construct
  source 1..410: mol_type = other DNA
agcatgaaagggatatacagattctgtacgcattgaagaagttctttgggtgcggtgttgtacgaaaaaaccacgatgatcgatatgaacttcggatccggaagaagtcttgcttgaagaaagtagtggaattcttcgaaaagcaccctctgaaaacgaagaagaacgttgacttcaagaagttcagaagaataatcctgatgatggaacggggagaacacctgacgaaagaaggtctaatcaagatcttagaaatcgccatggaaatgaacacaggtaaccacgagagactgcgacgagtccttgaagagatccggggactggatgaagatacagtccacccccattccgaaaggatgggataagggtgagcgaaattccttgtcgggtaagttccgacctgcatgaat

SEQ ID NO: 54 - DNA, 369 bp, synthetic construct
  source 1..369: mol_type = other DNA
ccccggtaaacggcggccgtaactataacggtcctaaggtagcattcgctgcctgcccacagggaaacctgtggggcaatacccggctgtatgcgggaaagcccttagagcccttcctacctgggggctgcggccagcccaggtaaaaatggaagggattgggtaatccgcaggaaaccccgatgagggggatcctcagagactgtacgccgggcatccagtccccgtgagaaggggtggaaatcttggatctcaagcctgattgggttgttggattcgtcgatggtgaaggttgtttctacgtgggtgttaatagaaatcgcaccatgaagacaggttaccaagttctccctgaattcaggattgttc

SEQ ID NO: 55 - DNA, 371 bp, synthetic construct
  source 1..371: mol_type = other DNA
agttctttgggtgcggtgttgtacgaaaaaaccacgatgatcgatatgaacttcggatccggaagaagtcttgcttgaagaaagtagtggaattcttcgaaaagcaccctctgaaaacgaagaagaacgttgacttcaagaagttcagaagaataatcctgatgatggaacggggagaacacctgacgaaagaaggtctaatcaagatcttagaaatcgccatggaaatgaacacaggtaaccacgagagactgcgacgagtccttgaagagatccggggactggatgaagatacagtccacccccattccgaaaggatgggataagggtgagcgaaattccttgtcgggtaagttccgacctgcatgaat

SEQ ID NO: 56 - DNA, 408 bp, synthetic construct
  source 1..408: mol_type = other DNA
ccccggtaaacggcggccgtaactataacggtcctaaggtagcattcgctgcctgcccacagggaaacctgtggggcaatacccggctgtatgcgggaaagcccttagagcccttcctacctgggggctgcggccagcccaggtaaaaatggaagggattgggtaatccgcaggaaaccccgatgagggggatcctcagagactgtacgccgggcatccagtccccgtgagaaggggtggaaatcttggatctcaagcctgattgggttgttggattcgtcgatggtgaaggttgtttctacgtgggtgttaatagaaatcgcaccatgaagacaggttaccaagttctccctgaattcaggattgttcagcatgaaagggatatacagattctgtacgcattgaaga

SEQ ID NO: 57 - DNA, 649 bp, synthetic construct
  source 1..649: mol_type = other DNA
cggccagcccaggtaaaaatggaagggattgggtaatccgcaggaaaccccgatgagggggatcctcagagactgtacgccgggcatccagtccccgtgagaaggggtggaaatcttggatctcaagcctgattgggttgttggattcgtcgatggtgaaggttgtttctacgtgggtgttaatagaaatcgcaccatgaagacaggttaccaagttctccctgaattcaggattgttcagcatgaaagggatatacagattctgtacgcattgaagaagttctttgggtgcggtgttgtacgaaaaaaccacgatgatcgatatgaacttcggatccggaagaagtcttgcttgaagaaagtagtggaattcttcgaaaagcaccctctgaaaacgaagaagaacgttgacttcaagaagttcagaagaataatcctgatgatggaacggggagaacacctgacgaaagaaggtctaatcaagatcttagaaatcgccatggaaatgaacacaggtaaccacgagagactgcgacgagtccttgaagagatccggggactggatgaagatacagtccacccccattccgaaaggatgggataagggtgagcgaaattccttgtcgggtaagttccgacctgcatgaat

SEQ ID NO: 58 - DNA, 130 bp, synthetic construct
  source 1..130: mol_type = other DNA
ccccggtaaacggcggccgtaactataacggtcctaaggtagcattcgctgcctgcccacagggaaacctgtggggcaatacccggctgtatgcgggaaagcccttagagcccttcctacctgggggctg

SEQ ID NO: 59 - DNA, 760 bp, synthetic construct
  source 1..760: mol_type = other DNA
cgaaattccttgtcgggtaaaaaattgccccgctaaactgtaaagtttagtgataaagtcagctcatatcgggggaaccctcctgctttttagcaaagggcaatcccgagggaagtcttaaatgaccccgtaacgactgatccgaaaggtgaggcacgcatttgtgtgcaatacgctgacttcttgcccttgggtttatactcaagaagtaagtgactatggagaatttatttatgtatttacatttagagccatggtatgtaagtggtttaacagaaggagaagggtgtttttcgatatcatttaacttcagaaaaaagttaaaaattggtattgaaacaagaccatctttttccatcacgttaaatcaaagagatttacctctcttaaaagagatacattcgttttttgaatgtggagcaattagattttcacgaggggatcgtacgtataaatatgaagtccgttccgtaaaagatcttgtgaagcgaataattccacacttcgataactatcctcttagaggaggtaaacaaaaagattttcgatatttttctgaaatctgtaaaaaaatacataccaattttcatttaaataaacaacatttaattgaaataataaaaatggcttatctgatgaatccatcaggtaaacgtaggcatgaaataaatgatctcctaaggttgcttggtgagaaaatggtatagtctactccctatggaaacataggaaagagtgaagttccgacctgcacgaatgg

SEQ ID NO: 60 - DNA, 270 bp, synthetic construct
  source 1..270: mol_type = other DNA
ctggcgaggctcaacgagtaagattgactaaacgcttaaaagttattcttactatgggcggtacgtaaagaaacttacgtatgtttacctgtcaaactcggggaagccaatagcgcggtaatcccgaaccaagctccagaaatggagaaggtgtagagactggaaggcaggtaccctaacagtaaagctgagggtaaagggacagtccagaccacaaactggttaatccaggcagtgaaaactgtagatggtaagcataacctacggcaa

SEQ ID NO: 61 - DNA, 284 bp, synthetic construct
  source 1..284: mol_type = other DNA
acggtagacgcagcggacttagaaaactgggcctcgatcgcgaaagggatcgagtggcagctctcaaactcagggaaacctaaaactttaaacattaaagtcatggcaatcctgagccaagctaaagctaaacaactaacagctttagaaggtgcagagactagacgggagctaccctaacggattcagccgagggtaaagggatagtccaattctcaacatcgcgattgttgatggcagcgaaagttgcagagagaatgaaaatccgctgactgtaaaggtcg

SEQ ID NO: 62 - DNA, 816 bp, synthetic construct
  source 1..816: mol_type = other DNA
ggtaaacggcggccgtaactataaagaccgttgtagttacggtaaaaaactcggctgtatgcgggaaactctggagtgccggtgggtaccacaggtgtggtaacaatcccacggagtgcgaaagcgccagacaacccgcaggaaactcatctaagttaaggagaattttccatgctggacgttaaaagaattccaccgaaaataggttactaccttggcaggctttgcagacggagaagggagtttcatggttgttgtaagaaagaaagatgattataaaagtggttggaagatatctgtagctttcaatgtctcgaataaagataaggtagtgcttgcactttttaaaaggtatttgaactgtggaactctccgtcagcgtaaagatggtgtgtggtactatgaagtaggtaatttcaacgcgattgtggaaaatgtgatacctttctttgacagattcagatttctttctgcagccaagagaaattcatattcaaaattcaaaaaagttgtagaaataattggaagatctgaacatacgacaaaggaaggcattgaaaagatattatctttgaggaatcaaatgagtaataatcggtcaaagcgaaaacacaccgatcaggaagttttgggtagcttagatgaggatcctcagagaccatacgccgagcatcacatgggtttgaccccaaacggggatgcgccgccgacccatggatgatgatatggtccaatcctatggtaacatagggcctaaaatgggatagcctcaattgaggtgaatgaagtattaacgaacggtcctaaggtagcgaa

SEQ ID NO: 63 - DNA, 103 bp, synthetic construct
  source 1..103: mol_type = other DNA
cgtaaacggccacaagttcagcgtgtctggcgaggcgaaattccttgtcgggtaagttccgacctgcacgaatggcctacggcaagctgaccctgaagttcat

SEQ ID NO: 64 - DNA, 96 bp, synthetic construct
  source 1..96: mol_type = other DNA
gcgacgtaaacggccacaagttcagcgtgtctggcgaggctggcgaggctcataacctacggcaacctacggcaagctgaccctgaagttcatctg

SEQ ID NO: 65 - DNA, 110 bp, synthetic construct
  source 1..110: mol_type = other DNA
gcgacgtaaacggccacaagttcagcgtgtctggcgaggacggtagacgcagcggacttaaaatccgctgactgtaaaggtcgcctacggcaagctgaccctgaagttca

SEQ ID NO: 66 - DNA, 111 bp, synthetic construct
  source 1..111: mol_type = other DNA
taaacggccacaagttcagcgtgtctggcgaggggtaaacggcggccgtaactataacggtcctaaggtagcgaacctacggcaagctgaccctgaagttcatctgcacca

SEQ ID NO: 67 - DNA, 447 bp, synthetic construct
  source 1..447: mol_type = other DNA
aaaaaagttaaaaattggtattgaaacaagaccatctttttccatcacgttaaatcaaagagatttacctctcttaaaagagatacattcgttttttgaatgtggagcaattagattttcacgaggggatcgtacgtataaatatgaagtccgttccgtaaaagatcttgtgaagcgaataattccacacttcgataactatcctcttagaggaggtaaacaaaaagattttcgatatttttctgaaatctgtaaaaaaatacataccaattttcatttaaataaacaacatttaattgaaataataaaaatggcttatctgatgaatccatcaggtaaacgtaggcatgaaataaatgatctcctaaggttgcttggtgagaaaatggtatagtctactccctatggaaacataggaaagagtgaagttccgacctgcacgaatgg

SEQ ID NO: 68 - DNA, 313 bp, synthetic construct
  source 1..313: mol_type = other DNA
cgaaattccttgtcgggtaaaaaattgccccgctaaactgtaaagtttagtgataaagtcagctcatatcgggggaaccctcctgctttttagcaaagggcaatcccgagggaagtcttaaatgaccccgtaacgactgatccgaaaggtgaggcacgcatttgtgtgcaatacgctgacttcttgcccttgggtttatactcaagaagtaagtgactatggagaatttatttatgtatttacatttagagccatggtatgtaagtggtttaacagaaggagaagggtgtttttcgatatcatttaacttcag

SEQ ID NO: 69 - DNA, 307 bp, synthetic construct
  source 1..307: mol_type = other DNA
aatatgaagtccgttccgtaaaagatcttgtgaagcgaataattccacacttcgataactatcctcttagaggaggtaaacaaaaagattttcgatatttttctgaaatctgtaaaaaaatacataccaattttcatttaaataaacaacatttaattgaaataataaaaatggcttatctgatgaatccatcaggtaaacgtaggcatgaaataaatgatctcctaaggttgcttggtgagaaaatggtatagtctactccctatggaaacataggaaagagtgaagttccgacctgcacgaatgg

SEQ ID NO: 70 - DNA, 453 bp, synthetic construct
  source 1..453: mol_type = other DNA
cgaaattccttgtcgggtaaaaaattgccccgctaaactgtaaagtttagtgataaagtcagctcatatcgggggaaccctcctgctttttagcaaagggcaatcccgagggaagtcttaaatgaccccgtaacgactgatccgaaaggtgaggcacgcatttgtgtgcaatacgctgacttcttgcccttgggtttatactcaagaagtaagtgactatggagaatttatttatgtatttacatttagagccatggtatgtaagtggtttaacagaaggagaagggtgtttttcgatatcatttaacttcagaaaaaagttaaaaattggtattgaaacaagaccatctttttccatcacgttaaatcaaagagatttacctctcttaaaagagatacattcgttttttgaatgtggagcaattagattttcacgaggggatcgtacgtata

SEQ ID NO: 71 - DNA, 199 bp, synthetic construct
  source 1..199: mol_type = other DNA
aacttacgtatgtttacctgtcaaactcggggaagccaatagcgcggtaatcccgaaccaagctccagaaatggagaaggtgtagagactggaaggcaggtaccctaacagtaaagctgagggtaaagggacagtccagaccacaaactggttaatccaggcagtgaaaactgtagatggtaagcataacctacggcaa

SEQ ID NO: 72 - DNA, 130 bp, synthetic construct
  source 1..130: mol_type = other DNA
aatggagaaggtgtagagactggaaggcaggtaccctaacagtaaagctgagggtaaagggacagtccagaccacaaactggttaatccaggcagtgaaaactgtagatggtaagcataacctacggcaa

SEQ ID NO: 73 - DNA, 130 bp, synthetic construct; identical to SEQ ID NO: 72
  source 1..130: mol_type = other DNA

SEQ ID NO: 74 - DNA, 140 bp, synthetic construct
  source 1..140: mol_type = other DNA
ctggcgaggctcaacgagtaagattgactaaacgcttaaaagttattcttactatgggcggtacgtaaagaaacttacgtatgtttacctgtcaaactcggggaagccaatagcgcggtaatcccgaaccaagctccaga

SEQ ID NO: 75 - DNA, 86 bp, synthetic construct
  source 1..86: mol_type = other DNA
aagctgagggtaaagggacagtccagaccacaaactggttaatccaggcagtgaaaactgtagatggtaagcataacctacggcaa

SEQ ID NO: 76 - DNA, 184 bp, synthetic construct
  source 1..184: mol_type = other DNA
ctggcgaggctcaacgagtaagattgactaaacgcttaaaagttattcttactatgggcggtacgtaaagaaacttacgtatgtttacctgtcaaactcggggaagccaatagcgcggtaatcccgaaccaagctccagaaatggagaaggtgtagagactggaaggcaggtaccctaacagta

SEQ ID NO: 77 - DNA, 54 bp, synthetic construct
  source 1..54: mol_type = other DNA
aactggttaatccaggcagtgaaaactgtagatggtaagcataacctacggcaa

SEQ ID NO: 78 - DNA, 216 bp, synthetic construct
  source 1..216: mol_type = other DNA
ctggcgaggctcaacgagtaagattgactaaacgcttaaaagttattcttactatgggcggtacgtaaagaaacttacgtatgtttacctgtcaaactcggggaagccaatagcgcggtaatcccgaaccaagctccagaaatggagaaggtgtagagactggaaggcaggtaccctaacagtaaagctgagggtaaagggacagtccagaccaca

SEQ ID NO: 79 - DNA, 149 bp, synthetic construct
  source 1..149: mol_type = other DNA
ctaacagctttagaaggtgcagagactagacgggagctaccctaacggattcagccgagggtaaagggatagtccaattctcaacatcgcgattgttgatggcagcgaaagttgcagagagaatgaaaatccgctgactgtaaaggtcg

SEQ ID NO: 80 - DNA, 135 bp, synthetic construct
  source 1..135: mol_type = other DNA
acggtagacgcagcggacttagaaaactgggcctcgatcgcgaaagggatcgagtggcagctctcaaactcagggaaacctaaaactttaaacattaaagtcatggcaatcctgagccaagctaaagctaaacaa

SEQ ID NO: 81 - DNA, 98 bp, synthetic construct
  source 1..98: mol_type = other DNA
cagccgagggtaaagggatagtccaattctcaacatcgcgattgttgatggcagcgaaagttgcagagagaatgaaaatccgctgactgtaaaggtcg

SEQ ID NO: 82 - DNA, 186 bp, synthetic construct
  source 1..186: mol_type = other DNA
acggtagacgcagcggacttagaaaactgggcctcgatcgcgaaagggatcgagtggcagctctcaaactcagggaaacctaaaactttaaacattaaagtcatggcaatcctgagccaagctaaagctaaacaactaacagctttagaaggtgcagagactagacgggagctaccctaacggatt

SEQ ID NO: 83 - DNA, 722 bp, synthetic construct
  source 1..722: mol_type = other DNA
gtgtggtaacaatcccacggagtgcgaaagcgccagacaacccgcaggaaactcatctaagttaaggagaattttccatgctggacgttaaaagaattccaccgaaaataggttactaccttggcaggctttgcagacggagaagggagtttcatggttgttgtaagaaagaaagatgattataaaagtggttggaagatatctgtagctttcaatgtctcgaataaagataaggtagtgcttgcactttttaaaaggtatttgaactgtggaactctccgtcagcgtaaagatggtgtgtggtactatgaagtaggtaatttcaacgcgattgtggaaaatgtgatacctttctttgacagattcagatttctttctgcagccaagagaaattcatattcaaaattcaaaaaagttgtagaaataattggaagatctgaacatacgacaaaggaaggcattgaaaagatattatctttgaggaatcaaatgagtaataatcggtcaaagcgaaaacacaccgatcaggaagttttgggtagcttagatgaggatcctcagagaccatacgccgagcatcacatgggtttgaccccaaacggggatgcgccgccgacccatggatgatgatatggtccaatcctatggtaacatagggcctaaaatgggatagcctcaattgaggtgaatgaagtattaacgaacggtcctaaggtagcgaa

SEQ ID NO: 84 - DNA, 94 bp, synthetic construct
  source 1..94: mol_type = other DNA
ggtaaacggcggccgtaactataaagaccgttgtagttacggtaaaaaactcggctgtatgcgggaaactctggagtgccggtgggtaccacag

SEQ ID NO: 85 - DNA, 480 bp, synthetic construct
  source 1..480: mol_type = other DNA
tgcactttttaaaaggtatttgaactgtggaactctccgtcagcgtaaagatggtgtgtggtactatgaagtaggtaatttcaacgcgattgtggaaaatgtgatacctttctttgacagattcagatttctttctgcagccaagagaaattcatattcaaaattcaaaaaagttgtagaaataattggaagatctgaacatacgacaaaggaaggcattgaaaagatattatctttgaggaatcaaatgagtaataatcggtcaaagcgaaaacacaccgatcaggaagttttgggtagcttagatgaggatcctcagagaccatacgccgagcatcacatgggtttgaccccaaacggggatgcgccgccgacccatggatgatgatatggtccaatcctatggtaacatagggcctaaaatgggatagcctcaattgaggtgaatgaagtattaacgaacggtcctaaggtagcgaa

SEQ ID NO: 86 - DNA, 336 bp, synthetic construct
  source 1..336: mol_type = other DNA
ggtaaacggcggccgtaactataaagaccgttgtagttacggtaaaaaactcggctgtatgcgggaaactctggagtgccggtgggtaccacaggtgtggtaacaatcccacggagtgcgaaagcgccagacaacccgcaggaaactcatctaagttaaggagaattttccatgctggacgttaaaagaattccaccgaaaataggttactaccttggcaggctttgcagacggagaagggagtttcatggttgttgtaagaaagaaagatgattataaaagtggttggaagatatctgtagctttcaatgtctcgaataaagataaggtagtgct

SEQ ID NO: 87 - DNA, 324 bp, synthetic construct
  source 1..324: mol_type = other DNA
ttcaaaattcaaaaaagttgtagaaataattggaagatctgaacatacgacaaaggaaggcattgaaaagatattatctttgaggaatcaaatgagtaataatcggtcaaagcgaaaacacaccgatcaggaagttttgggtagcttagatgaggatcctcagagaccatacgccgagcatcacatgggtttgaccccaaacggggatgcgccgccgacccatggatgatgatatggtccaatcctatggtaacatagggcctaaaatgggatagcctcaattgaggtgaatgaagtattaacgaacggtcctaaggtagcgaa

SEQ ID NO: 88 - DNA, 492 bp, synthetic construct
  source 1..492: mol_type = other DNA
ggtaaacggcggccgtaactataaagaccgttgtagttacggtaaaaaactcggctgtatgcgggaaactctggagtgccggtgggtaccacaggtgtggtaacaatcccacggagtgcgaaagcgccagacaacccgcaggaaactcatctaagttaaggagaattttccatgctggacgttaaaagaattccaccgaaaataggttactaccttggcaggctttgcagacggagaagggagtttcatggttgttgtaagaaagaaagatgattataaaagtggttggaagatatctgtagctttcaatgtctcgaataaagataaggtagtgcttgcactttttaaaaggtatttgaactgtggaactctccgtcagcgtaaagatggtgtgtggtactatgaagtaggtaatttcaacgcgattgtggaaaatgtgatacctttctttgacagattcagatttctttctgcagccaagagaaattcata

SEQ ID NO: 89 - DNA, 239 bp, synthetic construct
  source 1..239: mol_type = other DNA
aatcaaatgagtaataatcggtcaaagcgaaaacacaccgatcaggaagttttgggtagcttagatgaggatcctcagagaccatacgccgagcatcacatgggtttgaccccaaacggggatgcgccgccgacccatggatgatgatatggtccaatcctatggtaacatagggcctaaaatgggatagcctcaattgaggtgaatgaagtattaacgaacggtcctaaggtagcgaa

SEQ ID NO: 90 - DNA, 577 bp, synthetic construct
  source 1..577: mol_type = other DNA
ggtaaacggcggccgtaactataaagaccgttgtagttacggtaaaaaactcggctgtatgcgggaaactctggagtgccggtgggtaccacaggtgtggtaacaatcccacggagtgcgaaagcgccagacaacccgcaggaaactcatctaagttaaggagaattttccatgctggacgttaaaagaattccaccgaaaataggttactaccttggcaggctttgcagacggagaagggagtttcatggttgttgtaagaaagaaagatgattataaaagtggttggaagatatctgtagctttcaatgtctcgaataaagataaggtagtgcttgcactttttaaaaggtatttgaactgtggaactctccgtcagcgtaaagatggtgtgtggtactatgaagtaggtaatttcaacgcgattgtggaaaatgtgatacctttctttgacagattcagatttctttctgcagccaagagaaattcatattcaaaattcaaaaaagttgtagaaataattggaagatctgaacatacgacaaaggaaggcattgaaaagatattatctttgagg

SEQ ID NO: 91 - DNA, 39 bp, synthetic construct
  source 1..39: mol_type = other DNA
gccgggatcactctcggcatggacgagctgtacaagtaa

SEQ ID NO: 92 - DNA, 37 bp, synthetic construct
  source 1..37: mol_type = other DNA
gggcctgtgggtgggatcaacccacaggctgttttaa

SEQ ID NO: 93 - DNA, 88 bp, synthetic construct
  source 1..88: mol_type = other DNA
cgaaattccttgtcgggtaagttccgacctgcacgaatgggccggaaacgcaatagccgaaaaacaaaaaacaaaaaaaaaaaaaaaa

SEQ ID NO: 94 - DNA, 121 bp, synthetic construct
  source 1..121: mol_type = other DNA
aaaaaacaaaaaacaaaacggctattatgcgttaccggcctggcgaggctcataacctacggcaagccggaaacgcaatagccgaaaaacaaaaaacaaaaaaaaaaaaaaaaaaaaaaaa

SEQ ID NO: 95 - DNA, 124 bp, synthetic construct
  source 1..124: mol_type = other DNA
aaaaaacaaaaaacaaaacggctattatgcgttaccggcacggtagacgcagcggacttaaaatccgctgactgtaaaggtcggccggaaacgcaatagccgaaaaacaaaaaacaaaaaaaaa

SEQ ID NO: 96 - DNA, 140 bp, synthetic construct
  source 1..140: mol_type = other DNA
aaaaaacaaaaaacaaaacggctattatgcgttaccggcggtaaacggcggccgtaactataacggtcctaaggtagcgaagccggaaacgcaatagccgaaaaacaaaaaacaaaaaaaaaaaaaaaaaaaaaaaaaaa